European Patent Application EP 4 464 780 A1, published November 20, 2024. Title: NUCLEOTIDE AND USE THEREOF. Applicant: GUANGZHOU REFORGENE MEDICINE CO., LTD. Application CN PCT/CN2023/070867, filed January 6, 2023. The sequence listing filed with the application follows.

SEQUENCE LISTING (39 sequences)

SEQ ID NO: 1 - RNA, 191 nt, synthetic construct
  misc_feature 1..191: note = exon 13 3' sequence
  source 1..191: mol_type = other RNA
cagtgtgagcctcacaggtacaatttgaccattgacaattttcaacactgccagatgtgtgagtgtgattccttggggacattacctgggaccatttgtgacccaatcagtggccagtgcctgtgtgtgcctaatcgtcaaggaagaaggtgtaatcagtgtcaaccaggtaagaaagaaatgtattacat

SEQ ID NO: 2 - RNA, 11 nt, synthetic construct
  misc_feature 1..11: note = U7 specific Sm sequence RNA
  source 1..11: mol_type = other RNA
aatttgtctag

SEQ ID NO: 3 - DNA, 11 bp, synthetic construct
  misc_feature 1..11: note = U7 specific Sm sequence DNA
  source 1..11: mol_type = other DNA
aatttgtctag

SEQ ID NO: 4 - DNA, 11 bp, synthetic construct
  misc_feature 1..11: note = smOPT DNA
  source 1..11: mol_type = other DNA
aatttttggag

SEQ ID NO: 5 - RNA, 11 nt, synthetic construct
  misc_feature 1..11: note = smOPT RNA
  source 1..11: mol_type = other RNA
aatttttggag

SEQ ID NO: 6 - RNA, 31 nt, synthetic construct
  misc_feature 1..31: note = U7 stem region
  misc_feature 29: note = n = Thiophosphorylated skeleton and 2 '- methoxy modification
  misc_feature 30: note = n = Thiophosphorylated skeleton and 2 '- methoxy modification
  misc_feature 31: note = n = Thiophosphorylated skeleton and 2 '- methoxy modification
  source 1..31: mol_type = other RNA
caggttttctgacttcggtcggaaaacccct

SEQ ID NO: 7 - DNA, 13 bp, synthetic construct
  misc_feature 1..13: note = U7 snRNA gene 3' post sequence
  source 1..13: mol_type = other DNA
gtctacaatgaaa

SEQ ID NO: 8 - RNA, 24 nt, synthetic construct
  misc_feature 1..24: note = SnRNA 9 recognition domain
  source 1..24: mol_type = other RNA
agaaatttaaatccaaaattgcaa

SEQ ID NO: 9 - RNA, 24 nt, synthetic construct
  misc_feature 1..24: note = snRNA 19 recognition domain
  source 1..24: mol_type = other RNA
actgagccatggaggttacactgg

SEQ ID NO: 10 - RNA, 24 nt, synthetic construct
  misc_feature 1..24: note = snRNA 20+AON 20 recognition domain
  source 1..24: mol_type = other RNA
attgtacctgtgaggctcacactg

SEQ ID NO: 11 - RNA, 24 nt, synthetic construct
  misc_feature 1..24: note = snRNA 24+AON 24 recognition domain
  source 1..24: mol_type = other RNA
accttcttccttgacgattaggca

SEQ ID NO: 12 - RNA, 24 nt, synthetic construct
  misc_feature 1..24: note = snRNA 25+AON 25 recognition domain
  source 1..24: mol_type = other RNA
attacaccttcttccttgacgatt

SEQ ID NO: 13 - RNA, 27 nt, synthetic construct
  misc_feature 1..27: note = snRNA 26 recognition domain
  source 1..27: mol_type = other RNA
attacaccttcttccttgacgattagg

SEQ ID NO: 14 - RNA, 24 nt, synthetic construct
  misc_feature 1..24: note = snRNA 27 recognition domain
  source 1..24: mol_type = other RNA
actgattacaccttcttccttgac

SEQ ID NO: 15 - RNA, 24 nt, synthetic construct
  misc_feature 1..24: note = snRNA 28 recognition domain
  source 1..24: mol_type = other RNA
acatttctttcttacctggttgac

SEQ ID NO: 16 - RNA, 22 nt, synthetic construct
  misc_feature 1..22: note = snRNA 29 recognition domain
  source 1..22: mol_type = other RNA
acatttctttcttacctggttg

SEQ ID NO: 17 - RNA, 27 nt, synthetic construct
  misc_feature 1..27: note = snRNA 30 recognition domain
  source 1..27: mol_type = other RNA
acatttctttcttacctggttgacact

SEQ ID NO: 18 - RNA, 24 nt, synthetic construct
  misc_feature 1..24: note = snRNA 31+AON 31 recognition domain
  source 1..24: mol_type = other RNA
acatttctttcttacctggttgcc

SEQ ID NO: 19 - RNA, 27 nt, synthetic construct
  misc_feature 1..27: note = snRNA 32 recognition domain
  source 1..27: mol_type = other RNA
acatttctttcttacctggttgccact

SEQ ID NO: 20 - RNA, 24 nt, synthetic construct
  misc_feature 1..24: note = snRNA 33 recognition domain
  source 1..24: mol_type = other RNA
aatacatttctttcttacctggtt

SEQ ID NO: 21 - RNA, 24 nt, synthetic construct
  misc_feature 1..24: note = snRNA 34 recognition domain
  source 1..24: mol_type = other RNA
atgtaatacatttctttcttacct

SEQ ID NO: 22 - RNA, 66 nt, synthetic construct
  misc_feature 1..66: note = U7-snRNA#25 modification 1
  misc_feature 1: note = n = Thiophosphorylated skeleton and 2 '- methoxy modification
  misc_feature 2: note = n = Thiophosphorylated skeleton and 2 '- methoxy modification
  misc_feature 3: note = n = Thiophosphorylated skeleton and 2 '- methoxy modification
  misc_feature 64: note = n = Thiophosphorylated skeleton and 2 '- methoxy modification
  misc_feature 65: note = n = Thiophosphorylated skeleton and 2 '- methoxy modification
  misc_feature 66: note = n = Thiophosphorylated skeleton and 2 '- methoxy modification
  source 1..66: mol_type = other RNA
attacaccttcttccttgacgattaatttttggagcaggttttctgacttcggtcggaaaacccct

SEQ ID NO: 23 - RNA, 75 nt, synthetic construct
  misc_feature 1..75: note = U7-snRNA#25 modification 2
  misc_feature 1: note = n = Thiophosphorylated skeleton and 2 '- methoxy modification
  misc_feature 2: note = n = Thiophosphorylated skeleton and 2 '- methoxy modification
  misc_feature 3: note = n = Thiophosphorylated skeleton and 2 '- methoxy modification
  misc_feature 73: note = n = Thiophosphorylated skeleton and 2 '- methoxy modification
  misc_feature 74: note = n = Thiophosphorylated skeleton and 2 '- methoxy modification
  misc_feature 75: note = n = Thiophosphorylated skeleton and 2 '- methoxy modification
  source 1..75: mol_type = other RNA
actgattacaccttcttccttgacgattaggcaaatttttggagcaggttttctgacttcggtcggaaaacccct

SEQ ID NO: 24 - RNA, 69 nt, synthetic construct
  misc_feature 1..69: note = U7-snRNA#26 modification 1
  misc_feature 1: note = n = Thiophosphorylated skeleton and 2 '- methoxy modification
  misc_feature 2: note = n = Thiophosphorylated skeleton and 2 '- methoxy modification
  misc_feature 3: note = n = Thiophosphorylated skeleton and 2 '- methoxy modification
  misc_feature 67: note = n = Thiophosphorylated skeleton and 2 '- methoxy modification
  misc_feature 68: note = n = Thiophosphorylated skeleton and 2 '- methoxy modification
  misc_feature 69: note = n = Thiophosphorylated skeleton and 2 '- methoxy modification
  source 1..69: mol_type = other RNA
attacaccttcttccttgacgattaggaatttttggagcaggttttctgacttcggtcggaaaacccct

SEQ ID NO: 25 - RNA, 82 nt, synthetic construct
  misc_feature 1..82: note = U7-snRNA#26 modification 2
  misc_feature 1: note = n = Thiophosphorylated skeleton and 2 '- methoxy modification
  misc_feature 2: note = n = Thiophosphorylated skeleton and 2 '- methoxy modification
  misc_feature 3: note = n = Thiophosphorylated skeleton and 2 '- methoxy modification
  misc_feature 80: note = n = Thiophosphorylated skeleton and 2 '- methoxy modification
  misc_feature 81: note = n = Thiophosphorylated skeleton and 2 '- methoxy modification
  misc_feature 82: note = n = Thiophosphorylated skeleton and 2 '- methoxy modification
  source 1..82: mol_type = other RNA
attacaccttcttccttgacgattaggcacacacaggcacaatttttggagcaggttttctgacttcggtcggaaaacccct

SEQ ID NO: 26 - DNA, 336 bp, synthetic construct
  misc_feature 1..336: note = EGFPleft
  source 1..336: mol_type = other DNA
atggtgagcaagggcgaggagctgttcaccggggtggtgcccatcctggtcgagctggacggcgacgtaaacggccacaagttcagcgtgtccggcgagggcgagggcgatgccacctacggcaagctgaccctgaagttcatctgcaccaccggcaagctgcccgtgccctggcccaccctcgtgaccaccctgacctacggcgtgcagtgcttcagccgctaccccgaccacatgaagcagcacgacttcttcaagtccgccatgcccgaaggctacgtccaggagcgcaccatcttcttcaaggacgacggcaactacaagacccgcgccgag

SEQ ID NO: 27 - DNA, 384 bp, synthetic construct
  misc_feature 1..384: note = EGFPright
  source 1..384: mol_type = other DNA
gtgaagttcgagggcgacaccctggtgaaccgcatcgagctgaagggcatcgacttcaaggaggacggcaacatcctggggcacaagctggagtacaactacaacagccacaacgtctatatcatggccgacaagcagaagaacggcatcaaggtgaacttcaagatccgccacaacatcgaggacggcagcgtgcagctcgccgaccactaccagcagaacacccccatcggcgacggccccgtgctgctgcccgacaaccactacctgagcacccagtccgccctgagcaaagaccccaacgagaagcgcgatcacatggtcctgctggagttcgtgaccgccgccgggatcactctcggcatggacgagctgtacaagtaa

SEQ ID NO: 28 - DNA, 26 bp, synthetic construct
  misc_feature 1..26: note = hnRNP A1 snRNA 5' sequence
  source 1..26: mol_type = other DNA
ccgcaatatgatagggacttagggtg

SEQ ID NO: 29 - DNA, 22 bp, synthetic construct
  misc_feature 1..22: note = hnRNP A1 snRNA 3' sequence
  source 1..22: mol_type = other DNA
caccctaagtccctatcatatt

SEQ ID NO: 30 - skipped

SEQ ID NO: 31 - RNA, 93 nt, synthetic construct
  misc_feature 1..93: note = U7-hnRNP A1-snRNA
  misc_feature 1: note = n = Thiophosphorylated skeleton and 2 '- methoxy modification
  misc_feature 2: note = n = Thiophosphorylated skeleton and 2 '- methoxy modification
  misc_feature 3: note = n = Thiophosphorylated skeleton and 2 '- methoxy modification
  misc_feature 91: note = n = Thiophosphorylated skeleton and 2 '- methoxy modification
  misc_feature 92: note = n = Thiophosphorylated skeleton and 2 '- methoxy modification
  misc_feature 93: note = n = Thiophosphorylated skeleton and 2 '- methoxy modification
  source 1..93: mol_type = other RNA
accgcaatatgatagggacttagggtgattacaccttcttccttgacgattaatttttggagcaggttttctgacttcggtcggaaaacccct

SEQ ID NO: 32 - RNA, 20 nt, synthetic construct
  misc_feature 1..20: note = tail sequence
  source 1..20: mol_type = other RNA
tatgatagggacttagggtg

SEQ ID NO: 33 - DNA, 437 bp, synthetic construct
  misc_feature 1..437: note = U7-snRNA Gene expression box skeleton
  source 1..437: mol_type = other DNA
aagcttaacaacataggagctgtgattggctgttttcagccaatcagcactgactcatttgcatagcctttacaagcggtcacaaactcaagaaacgagcggttttaatagtcttttagaatattgtttatcgaaccgaataaggaactgtgctttgtgattcacatatcagtggaggggtgtggaaatggcaccttgatctcaccctcatcgaaagtggagttgatgtccttccctggctcgctacagacgcacttccgcagagaccaatgtgggtctcgaatttttggagcaggttttctgacttcggtcggaaaacccctcccaatttcactggtctacaatgaaagcaaaacagttctcttccccgctccccggtgtgtgagaggggctttgatccttctctggtttcctaggaaacgcgtatgtgcggccgc

SEQ ID NO: 34 - DNA, 21 bp, synthetic construct
  misc_feature 1..21: note = primer 1
  source 1..21: mol_type = other DNA
agcctttccgccaaggtgatc

SEQ ID NO: 35 - DNA, 21 bp, synthetic construct
  misc_feature 1..21: note = primer 2
  source 1..21: mol_type = other DNA
cacaacgttgcccagcaatgg

SEQ ID NO: 36 - RNA, 27 nt, synthetic construct
  misc_feature 1..27: note = snRNA 4 recognition domain
  source 1..27: mol_type = other RNA
atgatcacacctaagccctaaagataa

SEQ ID NO: 37 - RNA, 22 nt, synthetic construct
  misc_feature 1..22: note = snRNA 16 recognition domain
  source 1..22: mol_type = other RNA
acactggcagggctcacatcca

SEQ ID NO: 38 - RNA, 20 nt, synthetic construct
  misc_feature 1..20: note = Scramble recognition domain
  source 1..20: mol_type = other RNA
aggtgtagtcgaccatcgtg

SEQ ID NO: 39 - RNA, 64 nt, synthetic construct
  misc_feature 1..64: note = exon 13 3' sequence 2
  source 1..64: mol_type = other RNA
tgcctaatcgtcaaggaagaaggtgtaatcagtgtcaaccaggtaagaaagaaatgtattacat